European Patent Application EP 4 253 609 A1, published October 4, 2023. Title: CONSTRUCTION METHOD FOR AND APPLICATION OF NUCLEIC ACID MULTIMERIZATION-MEDIATED MULTIVALENT PROTEIN DRUG AND VACCINE. Applicant: ASSEMBLY MEDICINE, LLC. The sequence listing filed with the application follows.

SEQUENCE LISTING (279 sequences)

SEQ ID NO: 1 - DNA, 36 bp, Artificial Sequence
  nucleic acid single strand numbered S1 in sequence set 3-1
acacctggttgttggataaatcgttgaaggctagga

SEQ ID NO: 2 - DNA, 36 bp, Artificial Sequence
  nucleic acid single strand numbered S2 in sequence set 3-1
atcctagccttcaacgaaaaaactagagtccgccga

SEQ ID NO: 3 - DNA, 36 bp, Artificial Sequence
  nucleic acid single strand numbered S3 in sequence set 3-1
atcggcggactctagttaaaatccaacaaccaggtg

SEQ ID NO: 4 - DNA, 36 bp, Artificial Sequence
  nucleic acid single strand numbered S1 in sequence set 3-2
atgcgttgagttccagtaaaggcaacatcaccacat

SEQ ID NO: 5 - DNA, 36 bp, Artificial Sequence
  nucleic acid single strand numbered S2 in sequence set 3-2
aatgtggtgatgttgccaaatctgaatcctcgtgct

SEQ ID NO: 6 - DNA, 36 bp, Artificial Sequence
  nucleic acid single strand numbered S3 in sequence set 3-2
aagcacgaggattcagaaaaactggaactcaacgca

SEQ ID NO: 7 - DNA, 36 bp, Artificial Sequence
  nucleic acid single strand numbered S1 in sequence set 3-3
attccaatcgtcctgtgaaaagttccgctctgagtt

SEQ ID NO: 8 - DNA, 36 bp, Artificial Sequence
  nucleic acid single strand numbered S2 in sequence set 3-3
aaactcagagcggaactaaactggcagatggatgaa

SEQ ID NO: 9 - DNA, 36 bp, Artificial Sequence
  nucleic acid single strand numbered S3 in sequence set 3-3
attcatccatctgccagaaacacaggacgattggaa

SEQ ID NO: 10 - DNA, 36 bp, Artificial Sequence
  nucleic acid single strand numbered S1 in sequence set 3-4
acgaggcaagttctgtgaaaatgactaccaggtccg

SEQ ID NO: 11 - DNA, 36 bp, Artificial Sequence
  nucleic acid single strand numbered S2 in sequence set 3-4
acggacctggtagtcataaaatccactgacgctgaa

SEQ ID NO: 12 - DNA, 36 bp, Artificial Sequence
  nucleic acid single strand numbered S3 in sequence set 3-4
attcagcgtcagtggataaacacagaacttgcctcg

SEQ ID NO: 13 - DNA, 36 bp, Artificial Sequence
  nucleic acid single strand numbered S1 in sequence set 3-5
atagttcgttgctcggaaaaggcattgagaggacct

SEQ ID NO: 14 - DNA, 36 bp, Artificial Sequence
  nucleic acid single strand numbered S2 in sequence set 3-5
aaggtcctctcaatgccaaaatggtgatgtcgcttg

SEQ ID NO: 15 - DNA, 36 bp, Artificial Sequence
  nucleic acid single strand numbered S3 in sequence set 3-5
acaagcgacatcaccataaatccgagcaacgaacta

SEQ ID NO: 16 - DNA, 36 bp, Artificial Sequence
  nucleic acid single strand numbered S1 in sequence set 3-6
agtcgtgtgcttccaagaaatagccaggtgaggact

SEQ ID NO: 17 - DNA, 36 bp, Artificial Sequence
  nucleic acid single strand numbered S2 in sequence set 3-6
aagtcctcacctggctaaaaaacagcggagtgtcat

SEQ ID NO: 18 - DNA, 36 bp, Artificial Sequence
  nucleic acid single strand numbered S3 in sequence set 3-6
aatgacactccgctgttaaacttggaagcacacgac

SEQ ID NO: 19 - DNA, 36 bp, Artificial Sequence
  nucleic acid single strand numbered S1 in sequence set 3-7
aacgcatcgcttgatagaaaagaggagcacggttat

SEQ ID NO: 20 - DNA, 36 bp, Artificial Sequence
  nucleic acid single strand numbered S2 in sequence set 3-7
aataaccgtgctcctctaaagtaggcaatccaccat

SEQ ID NO: 21 - DNA, 36 bp, Artificial Sequence
  nucleic acid single strand numbered S3 in sequence set 3-7
aatggtggattgcctacaaactatcaagcgatgcgt

SEQ ID NO: 22 - DNA, 36 bp, Artificial Sequence
  nucleic acid single strand numbered S1 in sequence set 3-8
agtcgttccaccgaacaaaatggctctggtcattga

SEQ ID NO: 23 - DNA, 36 bp, Artificial Sequence
  nucleic acid single strand numbered S2 in sequence set 3-8
atcaatgaccagagccaaaaaatcgcacatctcagg

SEQ ID NO: 24 - DNA, 36 bp, Artificial Sequence
  nucleic acid single strand numbered S3 in sequence set 3-8
acctgagatgtgcgattaaatgttcggtggaacgac

SEQ ID NO: 25 - DNA, 36 bp, Artificial Sequence
  nucleic acid single strand numbered S1 in sequence set 3-9
agcggagtgaccatagtaaaaggcaggacattgttc

SEQ ID NO: 26 - DNA, 36 bp, Artificial Sequence
  nucleic acid single strand numbered S2 in sequence set 3-9
agaacaatgtcctgcctaaagtgctcgtcgtgaaga

SEQ ID NO: 27 - DNA, 36 bp, Artificial Sequence
  nucleic acid single strand numbered S3 in sequence set 3-9
atcttcacgacgagcacaaaactatggtcactccgc

SEQ ID NO: 28 - DNA, 36 bp, Artificial Sequence
  nucleic acid single strand numbered S1 in sequence set 3-10
aattggaccgctctactaaaatggcaccacagtcaa

SEQ ID NO: 29 - DNA, 36 bp, Artificial Sequence
  nucleic acid single strand numbered S2 in sequence set 3-10
attgactgtggtgccataaacaggctatcagcatcc

SEQ ID NO: 30 - DNA, 36 bp, Artificial Sequence
  nucleic acid single strand numbered S3 in sequence set 3-10
aggatgctgatagcctgaaaagtagagcggtccaat

SEQ ID NO: 31 - DNA, 36 bp, Artificial Sequence
  nucleic acid single strand numbered S1 in sequence set 3-11
accattgagccagtgataaaaaccgttgtgagttgc

SEQ ID NO: 32 - DNA, 36 bp, Artificial Sequence
  nucleic acid single strand numbered S2 in sequence set 3-11
agcaactcacaacggttaaatcgcacacctgtcgta

SEQ ID NO: 33 - DNA, 36 bp, Artificial Sequence
  nucleic acid single strand numbered S3 in sequence set 3-11
atacgacaggtgtgcgaaaaatcactggctcaatgg

SEQ ID NO: 34 - DNA, 36 bp, Artificial Sequence
  nucleic acid single strand numbered S1 in sequence set 3-12
aagtgaagaagcagcctaaagttgtcatcgcacacc

SEQ ID NO: 35 - DNA, 36 bp, Artificial Sequence
  nucleic acid single strand numbered S2 in sequence set 3-12
aggtgtgcgatgacaacaaaatgtcgtaaccgtgga

SEQ ID NO: 36 - DNA, 36 bp, Artificial Sequence
  nucleic acid single strand numbered S3 in sequence set 3-12
atccacggttacgacataaaaggctgcttcttcact

SEQ ID NO: 37 - DNA, 36 bp, Artificial Sequence
  nucleic acid single strand numbered S1 in sequence set 3-13
aatagcgtcttgagcctaaatggaggacataccgac

SEQ ID NO: 38 - DNA, 36 bp, Artificial Sequence
  nucleic acid single strand numbered S2 in sequence set 3-13
agtcggtatgtcctccaaaaggtcacagttgctgct

SEQ ID NO: 39 - DNA, 36 bp, Artificial Sequence
  nucleic acid single strand numbered S3 in sequence set 3-13
aagcagcaactgtgaccaaaaggctcaagacgctat

SEQ ID NO: 40 - DNA, 36 bp, Artificial Sequence
  nucleic acid single strand numbered S1 in sequence set 3-14
atgccgtgttcagattcaaatgtgcgtctggattga

SEQ ID NO: 41 - DNA, 36 bp, Artificial Sequence
  nucleic acid single strand numbered S2 in sequence set 3-14
atcaatccagacgcacaaaaagacaggtggtccgat

SEQ ID NO: 42 - DNA, 36 bp, Artificial Sequence
  nucleic acid single strand numbered S3 in sequence set 3-14
aatcggaccacctgtctaaagaatctgaacacggca

SEQ ID NO: 43 - DNA, 36 bp, Artificial Sequence
  nucleic acid single strand numbered S1 in sequence set 3-15
attcaggacagcgtcataaaaccgactggagcaact

SEQ ID NO: 44 - DNA, 36 bp, Artificial Sequence
  nucleic acid single strand numbered S2 in sequence set 3-15
aagttgctccagtcggtaaagatgccttcgtgtgag

SEQ ID NO: 45 - DNA, 36 bp, Artificial Sequence
  nucleic acid single strand numbered S3 in sequence set 3-15
actcacacgaaggcatcaaaatgacgctgtcctgaa

SEQ ID NO: 46 - DNA, 36 bp, Artificial Sequence
  nucleic acid single strand numbered S1 in sequence set 3-16
agcagccaaggttatctaaacaatgacacggaggat

SEQ ID NO: 47 - DNA, 36 bp, Artificial Sequence
  nucleic acid single strand numbered S2 in sequence set 3-16
aatcctccgtgtcattgaaagtgattcgcaccagac

SEQ ID NO: 48 - DNA, 36 bp, Artificial Sequence
  nucleic acid single strand numbered S3 in sequence set 3-16
agtctggtgcgaatcacaaaagataaccttggctgc

SEQ ID NO: 49 - DNA, 36 bp, Artificial Sequence
  nucleic acid single strand numbered S1 in sequence set 3-17
accaccgtgtatgacctaaaagtgacagcacatcgc

SEQ ID NO: 50 - DNA, 36 bp, Artificial Sequence
  nucleic acid single strand numbered S2 in sequence set 3-17
agcgatgtgctgtcactaaaacaggctctacgagga

SEQ ID NO: 51 - DNA, 36 bp, Artificial Sequence
  nucleic acid single strand numbered S3 in sequence set 3-17
atcctcgtagagcctgtaaaaggtcatacacggtgg

SEQ ID NO: 52 - DNA, 36 bp, Artificial Sequence
  nucleic acid single strand numbered S1 in sequence set 3-18
aactacggagcgaagataaatcctgaccaacttgct

SEQ ID NO: 53 - DNA, 36 bp, Artificial Sequence
  nucleic acid single strand numbered S2 in sequence set 3-18
aagcaagttggtcaggaaaagactggctgaacacga

SEQ ID NO: 54 - DNA, 36 bp, Artificial Sequence
  nucleic acid single strand numbered S3 in sequence set 3-18
atcgtgttcagccagtcaaaatcttcgctccgtagt

SEQ ID NO: 55 - DNA, 36 bp, Artificial Sequence
  nucleic acid single strand numbered S1 in sequence set 3-19
agttcctgatccagcctaaacatccttgtcttgcca

SEQ ID NO: 56 - DNA, 36 bp, Artificial Sequence
  nucleic acid single strand numbered S2 in sequence set 3-19
atggcaagacaaggatgaaacacgaccgcttagaag

SEQ ID NO: 57 - DNA, 36 bp, Artificial Sequence
  nucleic acid single strand numbered S3 in sequence set 3-19
acttctaagcggtcgtgaaaaggctggatcaggaac

SEQ ID NO: 58 - DNA, 36 bp, Artificial Sequence
  nucleic acid single strand numbered S1 in sequence set 3-20
atatcgcactccagcataaaccgtgtgaacatcagg

SEQ ID NO: 59 - DNA, 36 bp, Artificial Sequence
  nucleic acid single strand numbered S2 in sequence set 3-20
acctgatgttcacacggaaaagcctacgagacttgg

SEQ ID NO: 60 - DNA, 36 bp, Artificial Sequence
  nucleic acid single strand numbered S3 in sequence set 3-20
accaagtctcgtaggctaaaatgctggagtgcgata

SEQ ID NO: 61 - DNA, 32 bp, Artificial Sequence
  nucleic acid single strand numbered S1 in sequence set 4-1
aagcgtcgtgaatccaaatgagcctgccaatg

SEQ ID NO: 62 - DNA, 32 bp, Artificial Sequence
  nucleic acid single strand numbered S2 in sequence set 4-1
acattggcaggctcaaaaccgaagtcaacgct

SEQ ID NO: 63 - DNA, 32 bp, Artificial Sequence
  nucleic acid single strand numbered S3 in sequence set 4-1
aagcgttgacttcggaaaactatggacggcga

SEQ ID NO: 64 - DNA, 32 bp, Artificial Sequence
  nucleic acid single strand numbered S4 in sequence set 4-1
atcgccgtccatagtaaaggattcacgacgct

SEQ ID NO: 65 - DNA, 32 bp, Artificial Sequence
  nucleic acid single strand numbered S1 in sequence set 4-2
aatggcgagcaatccaaatgagcctggaccaa

SEQ ID NO: 66 - DNA, 32 bp, Artificial Sequence
  nucleic acid single strand numbered S2 in sequence set 4-2
attggtccaggctcaaaaccgaacgctgtgat

SEQ ID NO: 67 - DNA, 32 bp, Artificial Sequence
  nucleic acid single strand numbered S3 in sequence set 4-2
aatcacagcgttcggaaaactatcgtgcggca

SEQ ID NO: 68 - DNA, 32 bp, Artificial Sequence
  nucleic acid single strand numbered S4 in sequence set 4-2
atgccgcacgatagtaaaggattgctcgccat

SEQ ID NO: 69 - DNA, 32 bp, Artificial Sequence
  nucleic acid single strand numbered S1 in sequence set 4-3
atgaccacgcaatccaaatgagccaacctcca

SEQ ID NO: 70 - DNA, 32 bp, Artificial Sequence
  nucleic acid single strand numbered S2 in sequence set 4-3
atggaggttggctcaaaaccgaacagcagctt

SEQ ID NO: 71 - DNA, 32 bp, Artificial Sequence
  nucleic acid single strand numbered S3 in sequence set 4-3
aaagctgctgttcggaaaactatctgccgcct

SEQ ID NO: 72 - DNA, 32 bp, Artificial Sequence
  nucleic acid single strand numbered S4 in sequence set 4-3
aaggcggcagatagtaaaggattgcgtggtca

SEQ ID NO: 73 - DNA, 32 bp, Artificial Sequence
  nucleic acid single strand numbered S1 in sequence set 4-4
atgtcgcaccaatccaaatgagcaagcctcgt

SEQ ID NO: 74 - DNA, 32 bp, Artificial Sequence
  nucleic acid single strand numbered S2 in sequence set 4-4
aacgaggcttgctcaaaaccgaacgctgtcat

SEQ ID NO: 75 - DNA, 32 bp, Artificial Sequence
  nucleic acid single strand numbered S3 in sequence set 4-4
aatgacagcgttcggaaaactatgtggcggca

SEQ ID NO: 76 - DNA, 32 bp, Artificial Sequence
  nucleic acid single strand numbered S4 in sequence set 4-4
atgccgccacatagtaaaggattggtgcgaca

SEQ ID NO: 77 - DNA, 32 bp, Artificial Sequence
  nucleic acid single strand numbered S1 in sequence set 4-5
atgctggcacaatccaaatgagcgacgaggtt

SEQ ID NO: 78 - DNA, 32 bp, Artificial Sequence
  nucleic acid single strand numbered S2 in sequence set 4-5
aaacctcgtcgctcaaaaccgaagtgccagtt

SEQ ID NO: 79 - DNA, 32 bp, Artificial Sequence
  nucleic acid single strand numbered S3 in sequence set 4-5
aaactggcacttcggaaaactatgaggcggct

SEQ ID NO: 80 - DNA, 32 bp, Artificial Sequence
  nucleic acid single strand numbered S4 in sequence set 4-5
aagccgcctcatagtaaaggattgtgccagca

SEQ ID NO: 81 - DNA, 32 bp, Artificial Sequence
  nucleic acid single strand numbered S1 in sequence set 4-6
atgtcgcaccaatccaaatgagcaggttggca

SEQ ID NO: 82 - DNA, 32 bp, Artificial Sequence
  nucleic acid single strand numbered S2 in sequence set 4-6
atgccaacctgctcaaaaccgaacgctgtcaa

SEQ ID NO: 83 - DNA, 32 bp, Artificial Sequence
  nucleic acid single strand numbered S3 in sequence set 4-6
attgacagcgttcggaaaactatcagccgcct

SEQ ID NO: 84 - DNA, 32 bp, Artificial Sequence
  nucleic acid single strand numbered S4 in sequence set 4-6
aaggcggctgatagtaaaggattggtgcgaca

SEQ ID NO: 85 - DNA, 32 bp, Artificial Sequence
  nucleic acid single strand numbered S1 in sequence set 4-7
atgtggtcgcaatccaaatgagcacctgccaa

SEQ ID NO: 86 - DNA, 32 bp, Artificial Sequence
  nucleic acid single strand numbered S2 in sequence set 4-7
attggcaggtgctcaaaaccgaacgtgacgat

SEQ ID NO: 87 - DNA, 32 bp, Artificial Sequence
  nucleic acid single strand numbered S3 in sequence set 4-7
aatcgtcacgttcggaaaactatcaacgccgc

SEQ ID NO: 88 - DNA, 32 bp, Artificial Sequence
  nucleic acid single strand numbered S4 in sequence set 4-7
agcggcgttgatagtaaaggattgcgaccaca

SEQ ID NO: 89 - DNA, 32 bp, Artificial Sequence
  nucleic acid single strand numbered S1 in sequence set 4-8
aagcgtcgtcaatccaaatgagcacggcaatg

SEQ ID NO: 90 - DNA, 32 bp, Artificial Sequence
  nucleic acid single strand numbered S2 in sequence set 4-8
acattgccgtgctcaaaaccgaagtgaacgct

SEQ ID NO: 91 - DNA, 32 bp, Artificial Sequence
  nucleic acid single strand numbered S3 in sequence set 4-8
aagcgttcacttcggaaaactatggctcgcct

SEQ ID NO: 92 - DNA, 32 bp, Artificial Sequence
  nucleic acid single strand numbered S4 in sequence set 4-8
aaggcgagccatagtaaaggattgacgacgct

SEQ ID NO: 93 - DNA, 32 bp, Artificial Sequence
  nucleic acid single strand numbered S1 in sequence set 4-9
atgtggcgacaatccaaatgagcaagcctcca

SEQ ID NO: 94 - DNA, 32 bp, Artificial Sequence
  nucleic acid single strand numbered S2 in sequence set 4-9
atggaggcttgctcaaaaccgaagacgctgtt

SEQ ID NO: 95 - DNA, 32 bp, Artificial Sequence
  nucleic acid single strand numbered S3 in sequence set 4-9
aaacagcgtcttcggaaaactatcgtgcggca

SEQ ID NO: 96 - DNA, 32 bp, Artificial Sequence
  nucleic acid single strand numbered S4 in sequence set 4-9
atgccgcacgatagtaaaggattgtcgccaca

SEQ ID NO: 97 - DNA, 32 bp, Artificial Sequence
  nucleic acid single strand numbered S1 in sequence set 4-10
atgctgccacaatccaaatgagcctggaacca

SEQ ID NO: 98 - DNA, 32 bp, Artificial Sequence
  nucleic acid single strand numbered S2 in sequence set 4-10
atggttccaggctcaaaaccgaacgcagtcat

SEQ ID NO: 99 - DNA, 32 bp, Artificial Sequence
  nucleic acid single strand numbered S3 in sequence set 4-10
aatgactgcgttcggaaaactatcgccgctct

SEQ ID NO: 100 - DNA, 32 bp, Artificial Sequence
  nucleic acid single strand numbered S4 in sequence set 4-10
aagagcggcgatagtaaaggattgtggcagca

SEQ ID NO: 101 - DNA, 32 bp, Artificial Sequence
  nucleic acid single strand numbered S1 in sequence set 4-11
atgcgtcgtcaatccaaatgagcttggcaagg

SEQ ID NO: 102 - DNA, 32 bp, Artificial Sequence
  nucleic acid single strand numbered S2 in sequence set 4-11
accttgccaagctcaaaaccgaacgtgctgtt

SEQ ID NO: 103 - DNA, 32 bp, Artificial Sequence
  nucleic acid single strand numbered S3 in sequence set 4-11
aaacagcacgttcggaaaactatggagcggct

SEQ ID NO: 104 - DNA, 32 bp, Artificial Sequence
  nucleic acid single strand numbered S4 in sequence set 4-11
aagccgctccatagtaaaggattgacgacgca

SEQ ID NO: 105 - DNA, 32 bp, Artificial Sequence
  nucleic acid single strand numbered S1 in sequence set 4-12
aactgccagcaatccaaatgagcctcgttcca

SEQ ID NO: 106 - DNA, 32 bp, Artificial Sequence
  nucleic acid single strand numbered S2 in sequence set 4-12
atggaacgaggctcaaaaccgaagttggcagt

SEQ ID NO: 107 - DNA, 32 bp, Artificial Sequence
  nucleic acid single strand numbered S3 in sequence set 4-12
aactgccaacttcggaaaactatcgccgcttg

SEQ ID NO: 108 - DNA, 32 bp, Artificial Sequence
  nucleic acid single strand numbered S4 in sequence set 4-12
acaagcggcgatagtaaaggattgctggcagt

SEQ ID NO: 109 - DNA, 32 bp, Artificial Sequence
  nucleic acid single strand numbered S1 in sequence set 4-13
atgcgtcgtcaatccaaatgagcctccaggtt

SEQ ID NO: 110 - DNA, 32 bp, Artificial Sequence
  nucleic acid single strand numbered S2 in sequence set 4-13
aaacctggaggctcaaaaccgaatgacacgct

SEQ ID NO: 111 - DNA, 32 bp, Artificial Sequence
  nucleic acid single strand numbered S3 in sequence set 4-13
aagcgtgtcattcggaaaactatggcggcagt

SEQ ID NO: 112 - DNA, 32 bp, Artificial Sequence
  nucleic acid single strand numbered S4 in sequence set 4-13
aactgccgccatagtaaaggattgacgacgca

SEQ ID NO: 113 - DNA, 32 bp, Artificial Sequence
  nucleic acid single strand numbered S1 in sequence set 4-14
aagcgtcgtgaatccaaatgagccatcgtcca

SEQ ID NO: 114 - DNA, 32 bp, Artificial Sequence
  nucleic acid single strand numbered S2 in sequence set 4-14
atggacgatggctcaaaaccgaatgtgctggt

SEQ ID NO: 115 - DNA, 32 bp, Artificial Sequence
  nucleic acid single strand numbered S3 in sequence set 4-14
aaccagcacattcggaaaactatgcggcaacc

SEQ ID NO: 116 - DNA, 32 bp, Artificial Sequence
  nucleic acid single strand numbered S4 in sequence set 4-14
aggttgccgcatagtaaaggattcacgacgct

SEQ ID NO: 117 - DNA, 30 bp, Artificial Sequence
  nucleic acid single strand numbered S1 in sequence set 4-15
attgccaggatgctgaatcacggtcggaca

SEQ ID NO: 118 - DNA, 30 bp, Artificial Sequence
  nucleic acid single strand numbered S2 in sequence set 4-15
atgtccgaccgtgatagtcgcagaaggcat

SEQ ID NO: 119 - DNA, 30 bp, Artificial Sequence
  nucleic acid single strand numbered S3 in sequence set 4-15
aatgccttctgcgacatagtacaacgccgc

SEQ ID NO: 120 - DNA, 30 bp, Artificial Sequence
  nucleic acid single strand numbered S4 in sequence set 4-15
agcggcgttgtactaacagcatcctggcaa

SEQ ID NO: 121 - DNA, 32 bp, Artificial Sequence
  nucleic acid single strand numbered S1 in sequence set 4-16
aggcgatcacaatccaaatgagcgtgttacgg

SEQ ID NO: 122 - DNA, 32 bp, Artificial Sequence
  nucleic acid single strand numbered S2 in sequence set 4-16
accgtaacacgctcaaaaccgaagtgccaatt

SEQ ID NO: 123 - DNA, 32 bp, Artificial Sequence
  nucleic acid single strand numbered S3 in sequence set 4-16
aaattggcacttcggaaaactatgcggctgct

SEQ ID NO: 124 - DNA, 32 bp, Artificial Sequence
  nucleic acid single strand numbered S4 in sequence set 4-16
aagcagccgcatagtaaaggattgtgatcgcc

SEQ ID NO: 125 - DNA, 30 bp, Artificial Sequence
  nucleic acid single strand numbered S1 in sequence set 4-17
atggtccaacacgctaagcctcaccgtctt

SEQ ID NO: 126 - DNA, 30 bp, Artificial Sequence
  nucleic acid single strand numbered S2 in sequence set 4-17
aaagacggtgaggctatcgcacaacctggt

SEQ ID NO: 127 - DNA, 30 bp, Artificial Sequence
  nucleic acid single strand numbered S3 in sequence set 4-17
aaccaggttgtgcgaatcggagtggcagaa

SEQ ID NO: 128 - DNA, 30 bp, Artificial Sequence
  nucleic acid single strand numbered S4 in sequence set 4-17
attctgccactccgaaagcgtgttggacca

SEQ ID NO: 129 - DNA, 30 bp, Artificial Sequence
  nucleic acid single strand numbered S1 in sequence set 4-18
aaccttggtgtgcgaaactcctggcagcaa

SEQ ID NO: 130 - DNA, 30 bp, Artificial Sequence
  nucleic acid single strand numbered S2 in sequence set 4-18
attgctgccaggagtaagcgtgtggttcca

SEQ ID NO: 131 - DNA, 30 bp, Artificial Sequence
  nucleic acid single strand numbered S3 in sequence set 4-18
atggaaccacacgctatgaggaccgtcgtt

SEQ ID NO: 132 - DNA, 30 bp, Artificial Sequence
  nucleic acid single strand numbered S4 in sequence set 4-18
aaacgacggtcctcaatcgcacaccaaggt

SEQ ID NO: 133 - DNA, 30 bp, Artificial Sequence
  nucleic acid single strand numbered S1 in sequence set 4-19
atgccaagtccgagaatgctgcgaactggt

SEQ ID NO: 134 - DNA, 30 bp, Artificial Sequence
  nucleic acid single strand numbered S2 in sequence set 4-19
aaccagttcgcagcaaagagcctgaaccgt

SEQ ID NO: 135 - DNA, 30 bp, Artificial Sequence
  nucleic acid single strand numbered S3 in sequence set 4-19
aacggttcaggctctaacgacgcttgacca

SEQ ID NO: 136 - DNA, 30 bp, Artificial Sequence
  nucleic acid single strand numbered S4 in sequence set 4-19
atggtcaagcgtcgtatctcggacttggca

SEQ ID NO: 137 - DNA, 30 bp, Artificial Sequence
  nucleic acid single strand numbered S1 in sequence set 4-20
aagcagcctcgttgaatcgccaagacacct

SEQ ID NO: 138 - DNA, 30 bp, Artificial Sequence
  nucleic acid single strand numbered S2 in sequence set 4-20
aaggtgtcttggcgaaagttgctccgacga

SEQ ID NO: 139 - DNA, 30 bp, Artificial Sequence
  nucleic acid single strand numbered S3 in sequence set 4-20
atcgtcggagcaactaagcggttctgtgga

SEQ ID NO: 140 - DNA, 30 bp, Artificial Sequence
  nucleic acid single strand numbered S4 in sequence set 4-20
atccacagaaccgctatcaacgaggctgct

SEQ ID NO: 141 - DNA, 32 bp, Artificial Sequence
  nucleic acid single strand numbered S1 in sequence set 5-1
atcaggcgacctcttaaaaccaccatcgttgc

SEQ ID NO: 142 - DNA, 40 bp, Artificial Sequence
  nucleic acid single strand numbered S2 in sequence set 5-1
agcaacgatggtggtaaaaatccaaatgagcgtgttacgg

SEQ ID NO: 143 - DNA, 32 bp, Artificial Sequence; identical to SEQ ID NO: 122
  nucleic acid single strand numbered S3 in sequence set 5-1

SEQ ID NO: 144 - DNA, 32 bp, Artificial Sequence; identical to SEQ ID NO: 123
  nucleic acid single strand numbered S4 in sequence set 5-1

SEQ ID NO: 145 - DNA, 40 bp, Artificial Sequence
  nucleic acid single strand numbered S5 in sequence set 5-1
aagcagccgcatagtaaaggattaaaaagaggtcgcctga

SEQ ID NO: 146 - DNA, 32 bp, Artificial Sequence
  nucleic acid single strand numbered S1 in sequence set 5-2
aggcgacgatgtcttaaaacctggttgctgga

SEQ ID NO: 147 - DNA, 40 bp, Artificial Sequence
  nucleic acid single strand numbered S2 in sequence set 5-2
atccagcaaccaggtaaaaatccaaatgagcgtgttacgg

SEQ ID NO: 148 - DNA, 32 bp, Artificial Sequence; identical to SEQ ID NO: 122
  nucleic acid single strand numbered S3 in sequence set 5-2

SEQ ID NO: 149 - DNA, 32 bp, Artificial Sequence; identical to SEQ ID NO: 123
  nucleic acid single strand numbered S4 in sequence set 5-2

SEQ ID NO: 150 - DNA, 40 bp, Artificial Sequence
  nucleic acid single strand numbered S5 in sequence set 5-2
aagcagccgcatagtaaaggattaaaaagacatcgtcgcc

SEQ ID NO: 151 - DNA, 32 bp, Artificial Sequence
  nucleic acid single strand numbered S1 in sequence set 5-3
atggaacctggtgctaaatgctcgcctgtcaa

SEQ ID NO: 152 - DNA, 40 bp, Artificial Sequence
  nucleic acid single strand numbered S2 in sequence set 5-3
attgacaggcgagcaaaaaatccaaatgagcgtgttacgg

SEQ ID NO: 153 - DNA, 32 bp, Artificial Sequence; identical to SEQ ID NO: 122
  nucleic acid single strand numbered S3 in sequence set 5-3

SEQ ID NO: 154 - DNA, 32 bp, Artificial Sequence; identical to SEQ ID NO: 123
  nucleic acid single strand numbered S4 in sequence set 5-3

SEQ ID NO: 155 - DNA, 40 bp, Artificial Sequence
  nucleic acid single strand numbered S5 in sequence set 5-3
aagcagccgcatagtaaaggattaaaagcaccaggttcca

SEQ ID NO: 156 - DNA, 32 bp, Artificial Sequence
  nucleic acid single strand numbered S1 in sequence set 5-4
atggtcaggcgacttaaaaggacgaggttgct

SEQ ID NO: 157 - DNA, 40 bp, Artificial Sequence
  nucleic acid single strand numbered S2 in sequence set 5-4
aagcaacctcgtcctaaaaatccaaatgagcgtgttacgg

SEQ ID NO: 158 - DNA, 32 bp, Artificial Sequence; identical to SEQ ID NO: 122
  nucleic acid single strand numbered S3 in sequence set 5-4

SEQ ID NO: 159 - DNA, 32 bp, Artificial Sequence; identical to SEQ ID NO: 123
  nucleic acid single strand numbered S4 in sequence set 5-4

SEQ ID NO: 160 - DNA, 40 bp, Artificial Sequence
  nucleic acid single strand numbered S5 in sequence set 5-4
aagcagccgcatagtaaaggattaaaaagtcgcctgacca

SEQ ID NO: 161 - DNA, 32 bp, Artificial Sequence
  nucleic acid single strand numbered S1 in sequence set 5-5
atgctggaccaccttaaatcagatggaggcga

SEQ ID NO: 162 - DNA, 40 bp, Artificial Sequence
  nucleic acid single strand numbered S2 in sequence set 5-5
atcgcctccatctgaaaaaatccaaatgagcgtgttacgg

SEQ ID NO: 163 - DNA, 32 bp, Artificial Sequence; identical to SEQ ID NO: 122
  nucleic acid single strand numbered S3 in sequence set 5-5

SEQ ID NO: 164 - DNA, 32 bp, Artificial Sequence; identical to SEQ ID NO: 123
  nucleic acid single strand numbered S4 in sequence set 5-5

SEQ ID NO: 165 - DNA, 40 bp, Artificial Sequence
  nucleic acid single strand numbered S5 in sequence set 5-5
aagcagccgcatagtaaaggattaaaaaggtggtccagca

SEQ ID NO: 166 - DNA, 32 bp, Artificial Sequence
  nucleic acid single strand numbered S1 in sequence set 5-6
aaacgtccaggagctaaatctcgtcgcctgaa

SEQ ID NO: 167 - DNA, 40 bp, Artificial Sequence
  nucleic acid single strand numbered S2 in sequence set 5-6
attcaggcgacgagaaaaaatccaaatgagcgtgttacgg

SEQ ID NO: 168 - DNA, 32 bp, Artificial Sequence; identical to SEQ ID NO: 122
  nucleic acid single strand numbered S3 in sequence set 5-6

SEQ ID NO: 169 - DNA, 32 bp, Artificial Sequence; identical to SEQ ID NO: 123
  nucleic acid single strand numbered S4 in sequence set 5-6

SEQ ID NO: 170 - DNA, 40 bp, Artificial Sequence
  nucleic acid single strand numbered S5 in sequence set 5-6
aagcagccgcatagtaaaggattaaaagctcctggacgtt

SEQ ID NO: 171 - DNA, 32 bp, Artificial Sequence
  nucleic acid single strand numbered S1 in sequence set 5-7
accacgaccattgctaaaaacttcaggcgacg

SEQ ID NO: 172 - DNA, 40 bp, Artificial Sequence
  nucleic acid single strand numbered S2 in sequence set 5-7
acgtcgcctgaagttaaaaatccaaatgagcgtgttacgg

SEQ ID NO: 173 - DNA, 32 bp, Artificial Sequence; identical to SEQ ID NO: 122
  nucleic acid single strand numbered S3 in sequence set 5-7

SEQ ID NO: 174 - DNA, 32 bp, Artificial Sequence; identical to SEQ ID NO: 123
  nucleic acid single strand numbered S4 in sequence set 5-7

SEQ ID NO: 175 - DNA, 40 bp, Artificial Sequence
  nucleic acid single strand numbered S5 in sequence set 5-7
aagcagccgcatagtaaaggattaaaagcaatggtcgtgg

SEQ ID NO: 176 - DNA, 32 bp, Artificial Sequence
  nucleic acid single strand numbered S1 in sequence set 5-8
aaggcgaggtcttcaaaatggttgctggacga

SEQ ID NO: 177 - DNA, 40 bp, Artificial Sequence
  nucleic acid single strand numbered S2 in sequence set 5-8
atcgtccagcaaccaaaaaatccaaatgagcgtgttacgg

SEQ ID NO: 178 - DNA, 32 bp, Artificial Sequence; identical to SEQ ID NO: 122
  nucleic acid single strand numbered S3 in sequence set 5-8

SEQ ID NO: 179 - DNA, 32 bp, Artificial Sequence; identical to SEQ ID NO: 123
  nucleic acid single strand numbered S4 in sequence set 5-8

SEQ ID NO: 180 - DNA, 40 bp, Artificial Sequence
  nucleic acid single strand numbered S5 in sequence set 5-8
aagcagccgcatagtaaaggattaaatgaagacctcgcct

SEQ ID NO: 181 - DNA, 32 bp, Artificial Sequence
  nucleic acid single strand numbered S1 in sequence set 5-9
atcaaggcgaccagtaaaaagctcctcgacga

SEQ ID NO: 182 - DNA, 40 bp, Artificial Sequence
  nucleic acid single strand numbered S2 in sequence set 5-9
atcgtcgaggagcttaaaaatccaaatgagcgtgttacgg

SEQ ID NO: 183 - DNA, 32 bp, Artificial Sequence; identical to SEQ ID NO: 122
  nucleic acid single strand numbered S3 in sequence set 5-9

SEQ ID NO: 184 - DNA, 32 bp, Artificial Sequence; identical to SEQ ID NO: 123
  nucleic acid single strand numbered S4 in sequence set 5-9

SEQ ID NO: 185 - DNA, 40 bp, Artificial Sequence
  nucleic acid single strand numbered S5 in sequence set 5-9
aagcagccgcatagtaaaggattaaaactggtcgccttga

SEQ ID NO: 186 - DNA, 32 bp, Artificial Sequence
  nucleic acid single strand numbered S1 in sequence set 5-10
attcaggcgactcctaaaagcacgacgatggt

SEQ ID NO: 187 - DNA, 40 bp, Artificial Sequence
  nucleic acid single strand numbered S2 in sequence set 5-10
aaccatcgtcgtgctaaaaatccaaatgagcgtgttacgg

SEQ ID NO: 188 - DNA, 32 bp, Artificial Sequence; identical to SEQ ID NO: 122
  nucleic acid single strand numbered S3 in sequence set 5-10

SEQ ID NO: 189 - DNA, 32 bp, Artificial Sequence; identical to SEQ ID NO: 123
  nucleic acid single strand numbered S4 in sequence set 5-10

SEQ ID NO: 190 - DNA, 40 bp, Artificial Sequence
  nucleic acid single strand numbered S5 in sequence set 5-10
aagcagccgcatagtaaaggattaaaaggagtcgcctgaa

SEQ ID NO: 191 - DNA, 32 bp, Artificial Sequence
  nucleic acid single strand numbered S1 in sequence set 5-11
aagcacctgcaatccaaatcgccaggacaagt

SEQ ID NO: 192 - DNA, 32 bp, Artificial Sequence
  nucleic acid single strand numbered S2 in sequence set 5-11
aacttgtcctggcgaaaatgagcaaccatgcc

SEQ ID NO: 193 - DNA, 32 bp, Artificial Sequence
  nucleic acid single strand numbered S3 in sequence set 5-11
aggcatggttgctcaaaaccgaacgtcgtgat

SEQ ID NO: 194 - DNA, 32 bp, Artificial Sequence
  nucleic acid single strand numbered S4 in sequence set 5-11
aatcacgacgttcggaaaactatggagcggct

SEQ ID NO: 195 - DNA, 32 bp, Artificial Sequence
  nucleic acid single strand numbered S5 in sequence set 5-11
aagccgctccatagtaaaggattgcaggtgct

SEQ ID NO: 196 - DNA, 32 bp, Artificial Sequence
  nucleic acid single strand numbered S1 in sequence set 5-12
aacctgctgcaatccaaatcgccacctcaaga

SEQ ID NO: 197 - DNA, 32 bp, Artificial Sequence
  nucleic acid single strand numbered S2 in sequence set 5-12
atcttgaggtggcgaaaatgagcctggacgtt

SEQ ID NO: 198 - DNA, 32 bp, Artificial Sequence
  nucleic acid single strand numbered S3 in sequence set 5-12
aaacgtccaggctcaaaaccgaactggtgctt

SEQ ID NO: 199 - DNA, 32 bp, Artificial Sequence
  nucleic acid single strand numbered S4 in sequence set 5-12
aaagcaccagttcggaaaactatgccgctcct

SEQ ID NO: 200 - DNA, 32 bp, Artificial Sequence
  nucleic acid single strand numbered S5 in sequence set 5-12
aaggagcggcatagtaaaggattgcagcaggt

SEQ ID NO: 201 - DNA, 32 bp, Artificial Sequence
  nucleic acid single strand numbered S1 in sequence set 5-13
aagctggtgcaatccaaatcgcctcctgacaa

SEQ ID NO: 202 - DNA, 32 bp, Artificial Sequence
  nucleic acid single strand numbered S2 in sequence set 5-13
attgtcaggaggcgaaaatgagcaaggttggc

SEQ ID NO: 203 - DNA, 32 bp, Artificial Sequence
  nucleic acid single strand numbered S3 in sequence set 5-13
agccaaccttgctcaaaaccgaacgcagatgt

SEQ ID NO: 204 - DNA, 32 bp, Artificial Sequence
  nucleic acid single strand numbered S4 in sequence set 5-13
aacatctgcgttcggaaaactatggagcggca

SEQ ID NO: 205 - DNA, 32 bp, Artificial Sequence
  nucleic acid single strand numbered S5 in sequence set 5-13
atgccgctccatagtaaaggattgcaccagct

SEQ ID NO: 206 - DNA, 32 bp, Artificial Sequence
  nucleic acid single strand numbered S1 in sequence set 5-14
atgcacgcacaatccaaatcgccatcagaggt

SEQ ID NO: 207 - DNA, 32 bp, Artificial Sequence
  nucleic acid single strand numbered S2 in sequence set 5-14
aacctctgatggcgaaaatgagctgcctccat

SEQ ID NO: 208 - DNA, 32 bp, Artificial Sequence
  nucleic acid single strand numbered S3 in sequence set 5-14
aatggaggcagctcaaaaccgaacgtcgtcat

SEQ ID NO: 209 - DNA, 32 bp, Artificial Sequence
  nucleic acid single strand numbered S4 in sequence set 5-14
aatgacgacgttcggaaaactatcgagcggct

SEQ ID NO: 210 - DNA, 32 bp, Artificial Sequence
  nucleic acid single strand numbered S5 in sequence set 5-14
aagccgctcgatagtaaaggattgtgcgtgca

SEQ ID NO: 211 - DNA, 32 bp, Artificial Sequence
  nucleic acid single strand numbered S1 in sequence set 5-15
aagcgtcgtgaatccaaatcgccatcagacca

SEQ ID NO: 212 - DNA, 32 bp, Artificial Sequence
  nucleic acid single strand numbered S2 in sequence set 5-15
atggtctgatggcgaaaatgagcaaggctcgt

SEQ ID NO: 213 - DNA, 32 bp, Artificial Sequence
  nucleic acid single strand numbered S3 in sequence set 5-15
aacgagccttgctcaaaaccgaaccagcttgt

SEQ ID NO: 214 - DNA, 32 bp, Artificial Sequence
  nucleic acid single strand numbered S4 in sequence set 5-15
aacaagctggttcggaaaactatgcggcaggt

SEQ ID NO: 215 - DNA, 32 bp, Artificial Sequence
  nucleic acid single strand numbered S5 in sequence set 5-15
aacctgccgcatagtaaaggattcacgacgct

SEQ ID NO: 216 - DNA, 32 bp, Artificial Sequence
  nucleic acid single strand numbered S1 in sequence set 5-16
atcagcacgcaatccaaatcgccagttcaacc

SEQ ID NO: 217 - DNA, 32 bp, Artificial Sequence
  nucleic acid single strand numbered S2 in sequence set 5-16
aggttgaactggcgaaaatgagcaagcaggct

SEQ ID NO: 218 - DNA, 32 bp, Artificial Sequence
  nucleic acid single strand numbered S3 in sequence set 5-16
aagcctgcttgctcaaaaccgaacgtggtgtt

SEQ ID NO: 219 - DNA, 32 bp, Artificial Sequence
  nucleic acid single strand numbered S4 in sequence set 5-16
aaacaccacgttcggaaaactatggagcggca

SEQ ID NO: 220 - DNA, 32 bp, Artificial Sequence
  nucleic acid single strand numbered S5 in sequence set 5-16
atgccgctccatagtaaaggattgcgtgctga

SEQ ID NO: 221 - DNA, 32 bp, Artificial Sequence
  nucleic acid single strand numbered S1 in sequence set 5-17
aagctgcaccaatccaaatcgccagaaggtca

SEQ ID NO: 222 - DNA, 32 bp, Artificial Sequence
  nucleic acid single strand numbered S2 in sequence set 5-17
atgaccttctggcgaaaatgagcacgacgcat

SEQ ID NO: 223 - DNA, 32 bp, Artificial Sequence
  nucleic acid single strand numbered S3 in sequence set 5-17
aatgcgtcgtgctcaaaaccgaacaacctgct

SEQ ID NO: 224 - DNA, 32 bp, Artificial Sequence
  nucleic acid single strand numbered S4 in sequence set 5-17
aagcaggttgttcggaaaactatggagcggca

SEQ ID NO: 225 - DNA, 32 bp, Artificial Sequence
  nucleic acid single strand numbered S5 in sequence set 5-17
atgccgctccatagtaaaggattggtgcagct

SEQ ID NO: 226 - DNA, 32 bp, Artificial Sequence
  nucleic acid single strand numbered S1 in sequence set 5-18
aacgctcgtcaatccaaatcgcctcaggacaa

SEQ ID NO: 227 - DNA, 32 bp, Artificial Sequence
  nucleic acid single strand numbered S2 in sequence set 5-18
attgtcctgaggcgaaaatgagccaacgacct

SEQ ID NO: 228 - DNA, 32 bp, Artificial Sequence
  nucleic acid single strand numbered S3 in sequence set 5-18
aaggtcgttggctcaaaaccgaagctggtgtt

SEQ ID NO: 229 - DNA, 32 bp, Artificial Sequence
  nucleic acid single strand numbered S4 in sequence set 5-18
aaacaccagcttcggaaaactatgccgcacct

SEQ ID NO: 230 - DNA, 32 bp, Artificial Sequence
  nucleic acid single strand numbered S5 in sequence set 5-18
aaggtgcggcatagtaaaggattgacgagcgt

SEQ ID NO: 231 - DNA, 32 bp, Artificial Sequence
  nucleic acid single strand numbered S1 in sequence set 5-19
aagtgcgtcgaatccaaatcgccaagacctca

SEQ ID NO: 232 - DNA, 32 bp, Artificial Sequence
  nucleic acid single strand numbered S2 in sequence set 5-19
atgaggtcttggcgaaaatgagcaggctggaa

SEQ ID NO: 233 - DNA, 32 bp, Artificial Sequence
  nucleic acid single strand numbered S3 in sequence set 5-19
attccagcctgctcaaaaccgaagcaacgtgt

SEQ ID NO: 234 - DNA, 32 bp, Artificial Sequence
  nucleic acid single strand numbered S4 in sequence set 5-19
aacacgttgcttcggaaaactatgccgctcct

SEQ ID NO: 235 - DNA, 32 bp, Artificial Sequence
  nucleic acid single strand numbered S5 in sequence set 5-19
aaggagcggcatagtaaaggattcgacgcact

SEQ ID NO: 236 - DNA, 32 bp, Artificial Sequence
  nucleic acid single strand numbered S1 in sequence set 5-20
atcacgcagcaatccaaatcgccatcacaacg

SEQ ID NO: 237 - DNA, 32 bp, Artificial Sequence
  nucleic acid single strand numbered S2 in sequence set 5-20
acgttgtgatggcgaaaatgagcacgagcctt

SEQ ID NO: 238 - DNA, 32 bp, Artificial Sequence
  nucleic acid single strand numbered S3 in sequence set 5-20
aaaggctcgtgctcaaaaccgaaggttgcact

SEQ ID NO: 239 - DNA, 32 bp, Artificial Sequence
  nucleic acid single strand numbered S4 in sequence set 5-20
aagtgcaaccttcggaaaactatgccgctcca

SEQ ID NO: 240 - DNA, 32 bp, Artificial Sequence
  nucleic acid single strand numbered S5 in sequence set 5-20
atggagcggcatagtaaaggattgctgcgtga

SEQ ID NO: 241 - DNA, 36 bp, Artificial Sequence
  Trimer initial S1 sequence
agtgatccgaagtcgacaaacgtattagcgctcgat

SEQ ID NO: 242 - DNA, 36 bp, Artificial Sequence
  Trimer initial S2 sequence
aatcgagcgctaatacgaaagtgcaatgcgtcgatg

SEQ ID NO: 243 - DNA, 36 bp, Artificial Sequence
  Trimer initial S3 sequence
acatcgacgcattgcacaaagtcgacttcggatcac

SEQ ID NO: 244 - DNA, 36 bp, Artificial Sequence; identical to SEQ ID NO: 49
  Trimer optimized S1 sequence

SEQ ID NO: 245 - DNA, 36 bp, Artificial Sequence; identical to SEQ ID NO: 50
  Trimer optimized S2 sequence

SEQ ID NO: 246 - DNA, 36 bp, Artificial Sequence; identical to SEQ ID NO: 51
  Trimer optimized S3 sequence

SEQ ID NO: 247 - DNA, 32 bp, Artificial Sequence
  Tetramer initial S1 sequence
aacctggtacaatccaaatgagctacactagc

SEQ ID NO: 248 - DNA, 32 bp, Artificial Sequence
  Tetramer initial S2 sequence
agctagtgtagctcaaaaccgaagtatcgatt

SEQ ID NO: 249 - DNA, 32 bp, Artificial Sequence
  Tetramer initial S3 sequence
aaatcgatacttcggaaaactatagtgagttg

SEQ ID NO: 250 - DNA, 32 bp, Artificial Sequence
  Tetramer initial S4 sequence
acaactcactatagtaaaggattgtaccaggt

SEQ ID NO: 251 - DNA, 32 bp, Artificial Sequence; identical to SEQ ID NO: 121
  Tetramer optimized S1 sequence

SEQ ID NO: 252 - DNA, 32 bp, Artificial Sequence; identical to SEQ ID NO: 122
  Tetramer optimized S2 sequence

SEQ ID NO: 253 - DNA, 32 bp, Artificial Sequence; identical to SEQ ID NO: 123
  Tetramer optimized S3 sequence

SEQ ID NO: 254 - DNA, 32 bp, Artificial Sequence; identical to SEQ ID NO: 124
  Tetramer optimized S4 sequence

SEQ ID NO: 255 - DNA, 32 bp, Artificial Sequence
  Initial S1 sequence for the first conversion scheme of pentamers
atcacagagcgcgtaaaaacgccactcatgga

SEQ ID NO: 256 - DNA, 40 bp, Artificial Sequence
  Initial S2 sequence for the first conversion scheme of pentamers
atccatgagtggcgtaaaaatccaaatgagcgtgttacgg

SEQ ID NO: 257 - DNA, 32 bp, Artificial Sequence; identical to SEQ ID NO: 122
  Initial S3 sequence for the first conversion scheme of pentamers

SEQ ID NO: 258 - DNA, 32 bp, Artificial Sequence; identical to SEQ ID NO: 123
  Initial S4 sequence for the first conversion scheme of pentamers

SEQ ID NO: 259 - DNA, 40 bp, Artificial Sequence
  Initial S5 sequence for the first conversion scheme of pentamers
aagcagccgcatagtaaaggattaaatacgcgctctgtga

SEQ ID NO: 260 - DNA, 32 bp, Artificial Sequence; identical to SEQ ID NO: 186
  Optimized S1 sequence for the first conversion scheme of pentamers

SEQ ID NO: 261 - DNA, 40 bp, Artificial Sequence; identical to SEQ ID NO: 187
  Optimized S2 sequence for the first conversion scheme of pentamers

SEQ ID NO: 262 - DNA, 32 bp, Artificial Sequence; identical to SEQ ID NO: 122
  Optimized S3 sequence for the first conversion scheme of pentamers

SEQ ID NO: 263 - DNA, 32 bp, Artificial Sequence; identical to SEQ ID NO: 123
  Optimized S4 sequence for the first conversion scheme of pentamers

SEQ ID NO: 264 - DNA, 40 bp, Artificial Sequence; identical to SEQ ID NO: 190
  Optimized S5 sequence for the first conversion scheme of pentamers

SEQ ID NO: 265 - DNA, 32 bp, Artificial Sequence
  Initial S1 sequence for the second conversion scheme of pentamers
atgagtgcgcaatccaaatcgccagtcatgca

SEQ ID NO: 266 - DNA, 32 bp, Artificial Sequence
  Initial S2 sequence for the second conversion scheme of pentamers
atgcatgactggcgaaaatgagcgctcgttga

SEQ ID NO: 267 - DNA, 32 bp, Artificial Sequence
  Initial S3 sequence for the second conversion scheme of pentamers
atcaacgagcgctcaaaaccgaagtgccaact

SEQ ID NO: 268 - DNA, 32 bp, Artificial Sequence
  Initial S4 sequence for the second conversion scheme of pentamers
aagttggcacttcggaaaactatcgcgcgact

SEQ ID NO: 269 - DNA, 32 bp, Artificial Sequence
  Initial S5 sequence for the second conversion scheme of pentamers
aagtcgcgcgatagtaaaggattgcgcactca

SEQ ID NO: 270 - DNA, 32 bp, Artificial Sequence; identical to SEQ ID NO: 236
  Optimized S1 sequence for the second conversion scheme of pentamers

SEQ ID NO: 271 - DNA, 32 bp, Artificial Sequence; identical to SEQ ID NO: 237
  Optimized S2 sequence for the second conversion scheme of pentamers

SEQ ID NO: 272 - DNA, 32 bp, Artificial Sequence; identical to SEQ ID NO: 238
  Optimized S3 sequence for the second conversion scheme of pentamers

SEQ ID NO: 273 - DNA, 32 bp, Artificial Sequence; identical to SEQ ID NO: 239
  Optimized S4 sequence for the second conversion scheme of pentamers

SEQ ID NO: 274 - DNA, 32 bp, Artificial Sequence; identical to SEQ ID NO: 240
  Optimized S5 sequence for the second conversion scheme of pentamers

SEQ ID NO: 275 - DNA, 28 bp, Artificial Sequence
  PMO single strand 1 nucleic acid sequence
agcagcctcgttgaatcgccaagacacc

SEQ ID NO: 276 - DNA, 28 bp, Artificial Sequence
  PMO single strand 2 nucleic acid sequence
aggtgtcttggcgaaagttgctccgacg

SEQ ID NO: 277 - DNA, 28 bp, Artificial Sequence
  PMO single strand 3 nucleic acid sequence
acgtcggagcaactaagcggttctgtgg

SEQ ID NO: 278 - DNA, 28 bp, Artificial Sequence
  PMO single strand 4 nucleic acid sequence
accacagaaccgctatcaacgaggctgc

SEQ ID NO: 279 - protein, 124 aa, Artificial Sequence
  Amino acid sequence of anti-HSA nanoantibody mutant
HHHHHHAVQLVESGGGLVQPGNSLRLSCAASGFTFRSFGMSWVRQAPGKEPEWVSSISGSGSDTLYADSVKGRFTISRDNAKTTLYLQMNSLKPEDTAVYYCTIGGSLSRSSQGTQVTVSSGSC